European Patent Specification EP 3 991 755 B1, published August 21, 2024. Title: RNA AND NUCLEIC ACID DELIVERY SYSTEMS COMPRISING THE SAME. Applicant: LEMONEX INC. Application PCT/KR2021/008530. The sequence listing filed with the application follows.

SEQUENCE LISTING (49 sequences)

SEQ ID NO: 1 - RNA, 20 nt, Artificial Sequence
  siRNA
cacacauaugccauggugau

SEQ ID NO: 2 - RNA, 20 nt, Artificial Sequence
  siRNA
cacacauaugccauggugau

SEQ ID NO: 3 - RNA, 20 nt, Artificial Sequence
  siRNA
ugacuuaugagaacauggac

SEQ ID NO: 4 - RNA, 20 nt, Artificial Sequence
  siRNA
guccauguucucauaaguca

SEQ ID NO: 5 - RNA, 20 nt, Artificial Sequence
  siRNA
uggagacugcaguaaaggau

SEQ ID NO: 6 - RNA, 20 nt, Artificial Sequence
  siRNA
auccuuuacugcagucucca

SEQ ID NO: 7 - RNA, 20 nt, Artificial Sequence
  siRNA
agcugcuucugcaaucaaag

SEQ ID NO: 8 - DNA, 20 bp, Artificial Sequence
  siRNA
ctttgauugcagaagcagcu

SEQ ID NO: 9 - RNA, 19 nt, Artificial Sequence
  siRNA
ugauuccugcaagccagca

SEQ ID NO: 10 - RNA, 19 nt, Artificial Sequence
  siRNA
ugcuggcuugcaggaauca

SEQ ID NO: 11 - RNA, 24 nt, Artificial Sequence
  siRNA
agcugcuucugcaaucaaaguaau

SEQ ID NO: 12 - RNA, 24 nt, Artificial Sequence
  siRNA
auuacuuugauugcagaagcagcu

SEQ ID NO: 13 - DNA, 20 bp, Artificial Sequence
  CpG ODN
gggggacgatcgtcgggggg

SEQ ID NO: 14 - DNA, 24 bp, Artificial Sequence
  CpG ODN
tcgtcgttttgtcgttttgtcgtt

SEQ ID NO: 15 - DNA, 22 bp, Artificial Sequence
  CpG ODN
tcgtcgttttcggcgcgcgccg

SEQ ID NO: 16 - RNA, 20 nt, Artificial Sequence
  siRNA
ucaccauggcauaugugugg

SEQ ID NO: 17 - RNA, 20 nt, Artificial Sequence
  siRNA
ccacacauaugccaugguga

SEQ ID NO: 18 - RNA, 19 nt, Artificial Sequence
  siRNA
ucucauuucgugauggaga

SEQ ID NO: 19 - RNA, 19 nt, Artificial Sequence
  siRNA
ucuccaucacgaaaugaga

SEQ ID NO: 20 - RNA, 19 nt, Artificial Sequence
  siRNA
ucuggcuggaaaggcaacc

SEQ ID NO: 21 - RNA, 19 nt, Artificial Sequence
  siRNA
gguugccuuuccagccaga

SEQ ID NO: 22 - RNA, 17 nt, Artificial Sequence
  siRNA
ggucugguguaugaagg

SEQ ID NO: 23 - RNA, 20 nt, Artificial Sequence
  siRNA
ccacacauaugccaugguga

SEQ ID NO: 24 - DNA, 21 bp, Artificial Sequence
  primer
gatcctaataaccccctgact

SEQ ID NO: 25 - DNA, 18 bp, Artificial Sequence
  primer
cagcatctgctccaccag

SEQ ID NO: 26 - DNA, 21 bp, Artificial Sequence
  primer
tcactgccacccagaagactg

SEQ ID NO: 27 - DNA, 19 bp, Artificial Sequence
  primer
ggatcaccttgcccacagc

SEQ ID NO: 28 - DNA, 23 bp, Artificial Sequence
  primer
agctgcccgacgcatacagcccc

SEQ ID NO: 29 - DNA, 21 bp, Artificial Sequence
  primer
accccagggccaggtgtgcca

SEQ ID NO: 30 - DNA, 20 bp, Artificial Sequence
  primer
tggatttggacgcattggtc

SEQ ID NO: 31 - DNA, 21 bp, Artificial Sequence
  primer
tttgcactggtacgtgttgat

SEQ ID NO: 32 - DNA, 1849 bp, Homo sapiens
actgaggggcaccagaggagcagactacaagaatggcacacgctatggaaaactcctggacaatcagtaaagagtaccatattgatgaagaagtgggctttgctctgccaaatccacaggaaaatctacctgatttttataatgactggatgttcattgctaaacatctgcctgatctcatagagtctggccagcttcgagaaagagttgagaagttaaacatgctcagcattgatcatctcacagaccacaagtcacagcgccttgcacgtctagttctgggatgcatcaccatggcatatgtgtggggcaaaggtcatggagatgtccgtaaggtcttgccaagaaatattgctgttccttactgccaactctccaagaaactggaactgcctcctattttggtttatgcagactgtgtcttggcaaactggaagaaaaaggatcctaataagcccctgacttatgagaacatggacgttttgttctcatttcgtgatggagactgcagtaaaggattcttcctggtctctctattggtggaaatagcagctgcttctgcaatcaaagtaattcctactgtattcaaggcaatgcaaatgcaagaacgggacactttgctaaaggcgctgttggaaatagcttcttgcttggagaaagcccttcaagtgtttcaccaaatccacgatcatgtgaacccaaaagcatttttcagtgttcttcgcatatatttgtctggctggaaaggcaacccccagctatcagacggtctggtgtatgaagggttctgggaagacccaaaggagtttgcagggggcagtgcaggccaaagcagcgtctttcagtgctttgacgtcctgctgggcatccagcagactgctggtggaggacatgctgctcagttcctccaggacatgagaagatatatgccaccagctcacaggaacttcctgtgctcattagagtcaaatccctcagtccgtgagtttgtcctttcaaaaggtgatgctggcctgcgggaagcttatgacgcctgtgtgaaagctctggtctccctgaggagctaccatctgcaaatcgtgactaagtacatcctgattcctgcaagccagcagccaaaggagaataagacctctgaagacccttcaaaactggaagccaaaggaactggaggcactgatttaatgaatttcctgaagactgtaagaagtacaactgagaaatcccttttgaaggaaggttaatgtaacccaacaagagcacattttatcatagcagagacatctgtatgcattcctgtcattacccattgtaacagagccacaaactaatactatgcaatgttttaccaataatgcaatacaaaagacctcaaaatacctgtgcatttcttgtaggaaaacaacaaaaggtaattatgtgtaattatactagaagttttgtaatctgtatcttatcattggaataaaatgacattcaataaataaaaatgcataagatatattctgtcggctgggcgcggtggctcacgcctgtaatcccagcactttgggaggccgaggcgggcggatcacaaggtcaggagatcgagaccatcttggctaacacggtgaaaccccgtctctactaaaaatacaaaaaattagccgggcgcggtggcgggcacctgtagtcccagctactcgggaggctgaggcaggagaatggcgtgaacctgggaggcggagcttgcagtgagccaagattgtgccactgcaatccggcctgggctaaagagcgggactccgtctcaaaaaaaaaaaaaaaaagatatattctgtcataataaataaaaatgcataagatataa

SEQ ID NO: 33 - DNA, 1473 bp, Canis familiaris
gtggtcattggctgtggcaacctttataataagtagaggctctgaaactctatcagaactaaggaccaaaagaggagactgcaagcatggaagatgatggaatacttcttatggaaagtcctcagagaatttttgaaaaataccatatagatgaagagatgggcttcgctttgccaaatccactggagaagctacctccgccttatgatgaatggatttccattgctaaaaatctgcctgaactgattaagaaaaatgaactacgtaaaaaagttgatgagttaaaaattctcagtattgatggccttagtggacacaagttgcagcgccttgcacgtctggctctggggtatatcaccatggcatatgtgtggaatcaaggtgatggagatgttcgaaaggtcttgccacagaatattgctattccttactgtgaactctctgagaagctgggtctgcctcctattctggtttatgcagactgtgtcttagcaaactggaagaaaaaggatcccaatgggcctatgacttatgagaacatggacattctcttctggtttcctggtggagactgcagtaaaggatttttcctggtttcactattggtggaattagcagctgcttctgcaatcaaagtaattcccaatttattaaaggcagttaaaaatcaggacgaggtcactttgaagaaggcactgcattatatagcttcttgtctgcaccgagcccataaagagtttgaagaagttcataaacatgtggacccaagcacgtttttcaaagttcttcgcatatacttgtctggttggaaaggcaactccaaactgccagagggtttgaagtatgaaggtttctgggaaaacccaaaagagtttgcaggaggcagtgcagcccaaagcagcatctttcaatgctttgacattctgctgggcatccagcagtgttctggtgaagaattcgctgctgaattcctccaggaaatgagaaactatatgcccccagctcaccgggactttcttctcttgttaaagtcaggcccctcagtccgggagtttgttcgttcaagagatgatgttgaactgaaggcagattataatgagtgtgtgaaagctatggtctccctgagaaaatatcacttgaagatagtagctaagtacattgtgattcctgcaagccagcagcccaagaataatcaagcatctgaagaatcatcggaacaaaaaaataaaggaactggaggcactaatgccatggatttcctgaagagtgtaagaactacaactgagaaattcctgctgatagatcattaatgtaactcaaacaagggcacattttgtcaagatgaagatgtctgtatatattagtgtcactgctcatgatatcagacccatgaattaatagtacacaacaatgttttttttttacaacaatgttttaatagtacttataaaagatttcaaaatatttttccaa

SEQ ID NO: 34 - RNA, 24 nt, Homo sapiens
agcugcuucugcaaucaaaguaau

SEQ ID NO: 35 - RNA, 24 nt, Homo sapiens
auuacuuugauugcagaagcagcu

SEQ ID NO: 36 - RNA, 19 nt, Rattus norvegicus
gggcuucuuccucgucucu

SEQ ID NO: 37 - RNA, 19 nt, Rattus norvegicus
agagacgaggaagaagccc

SEQ ID NO: 38 - DNA, 20 bp, Homo sapiens
gggggacgatcgtcgggggg

SEQ ID NO: 39 - DNA, 20 bp, Rattus norvegicus
ggggtcaacgttgagggggg

SEQ ID NO: 40 - DNA, 20 bp, Homo sapiens
atcaccatggcatatgtgtg

SEQ ID NO: 41 - DNA, 20 bp, Homo sapiens
tgacttatgagaacatggac

SEQ ID NO: 42 - DNA, 20 bp, Homo sapiens
tggagactgcagtaaaggat

SEQ ID NO: 43 - DNA, 20 bp, Homo sapiens
agctgcttctgcaatcaaag

SEQ ID NO: 44 - DNA, 24 bp, Homo sapiens
agctgcttctgcaatcaaagtaat

SEQ ID NO: 45 - DNA, 24 bp, Homo sapiens
auuacuuugauugcagaagcagcu

SEQ ID NO: 46 - DNA, 20 bp, Homo sapiens
tcaccatggcatatgtgtgg

SEQ ID NO: 47 - DNA, 19 bp, Homo sapiens
tctcatttcgtgatggaga

SEQ ID NO: 48 - DNA, 19 bp, Homo sapiens
tctggctggaaaggcaacc

SEQ ID NO: 49 - DNA, 17 bp, Homo sapiens
ggtctggtgtatgaagg